European Patent Application EP 4 696 770 A1, published February 18, 2026. Title: LEVILACTOBACILLUS BREVIS AND USE THEREOF. Applicant: IBIOME BIOTECHNOLOGY CO., LTD. Application EP. The sequence listing filed with the application follows.

SEQUENCE LISTING (7 sequences)

SEQ ID NO: 1 - DNA, 1430 bp, Levilactobacillus brevis
  source 1..1430: mol_type = genomic DNA
ggctgactcccgaaggttatctcaccggctttgggtgttacaaactctcatggtgtgacgggcggtgtgtacaaggcccgggaacgtattcaccgcggcatgctgatccgcgattactagcgattccaacttcatgtaggcgagttgcagcctacaatccgaactgagaacggctttaagagattagcttagcctcacgacttcgcaactcgttgtaccgtccattgtagcacgtgtgtagcccaggtcataaggggcatgatgatttgacgtcatccccaccttcctccggtttgtcaccggcagtctcaccagagtgcccaactgaatgctggcaactgataataagggttgcgctcgttgcgggacttaacccaacatctcacgacacgagctgacgacaaccatgcaccacctgtcattctgtccccgaagggaacgtcttatctctaagattggcagaagatgtcaagacctggtaaggttcttcgcgtagcttcgaattaaaccacatgctccaccgcttgtgcgggcccccgtcaattcctttgagtttcaaccttgcggtcgtactccccaggcggagtgcttaatgcgttagctgcagcactgaagggcggaaaccctccaacacttagcactcatcgtttacggcatggactaccagggtatctaatcctgttcgctacccatgctttcgagcctcagcgtcagttacagactagacagccgccttcgccactggtgttcttccatatatctacgcattccaccgctacacatggagttccactgtcctcttctgcactcaagtctcccagtttccgatgcacttctccggttaagccgaaggctttcacatcagacttaaaaaaccgcctgcgctcgctttacgcccaataaatccggacaacgcttgccacctacgtattaccgcggctgctggcacgtagttagccgtggctttctggttaaataccgtcaacccttgaacagttactctcaaaggtgttcttctttaacaacagagttttacgagccgaaacccttcttcactcacgcggcattgctccatcagactttcgtccattgtggaagattccctactgctgcctcccgtaggagtttgggccgtgtctcagtcccaatgtggccgattaccctctcaggtcggctacgtatcatcgtcttggtgggcctttacctcaccaactaactaatacgccgcgggatcatccagaagtgatagccgaagccacctttcaaacaaaatccatgcggattttgttgttatacggtattagcacctgtttccaagtgttatcccctgcttctgggcagattccccacgtgttactcaccagttcgccactcgcttcattgttgaaatcagtgcaagcacgtcattcaacggaagctcgttcgactgc

SEQ ID NO: 2 - DNA, 20 bp, synthetic construct
  source 1..20: mol_type = other DNA
agagtttgatcctggctcag

SEQ ID NO: 3 - DNA, 19 bp, synthetic construct
  source 1..19: mol_type = other DNA
ggttaccttgttacgactt

SEQ ID NO: 4 - DNA, 18 bp, synthetic construct
  source 1..18: mol_type = other DNA
aaacaactgtattcccca

SEQ ID NO: 5 - DNA, 20 bp, synthetic construct
  source 1..20: mol_type = other DNA
caactaataggatcaccccc

SEQ ID NO: 6 - DNA, 20 bp, synthetic construct
  source 1..20: mol_type = other DNA
agagtttgatcctggctcag

SEQ ID NO: 7 - DNA, 19 bp, synthetic construct
  source 1..19: mol_type = other DNA
ggttaccttgttacgactt